European Patent Specification EP 3 363 913 B1, published June 7, 2023. Title: Procede optique de suivi de l'amplification in-vitro d'une sequence de nucleotides. Applicant: Commissariat a l'Energie Atomique et aux Energies Alternatives. The sequence listing filed with the application follows.

SEQUENCE LISTING (6 sequences)

SEQ ID NO: 1 - DNA, 18 bp, Escherichia coli
gccatctcctgatgacgc

SEQ ID NO: 2 - DNA, 18 bp, Escherichia coli
atttaccgcagccagacg

SEQ ID NO: 3 - DNA, 40 bp, Escherichia coli
ctggggcgaggtcgtggtattccgacaaacaccacgaatt

SEQ ID NO: 4 - DNA, 42 bp, Escherichia coli
cattttgcagctgtacgctcgcagcccatcatgaatgttgct

SEQ ID NO: 5 - DNA, 24 bp, Escherichia coli
ctttgtaacaacctgtcatcgaca

SEQ ID NO: 6 - DNA, 25 bp, Escherichia coli
atcaatctcgatatccatgaaggtg